European Patent Specification EP 3 762 049 B1, published April 10, 2024. Title: METHODS AND KITS FOR PRODUCING A FIBRIN MATRIX. Applicant: Vogt, Lorenz Irvine, Alistair Simpson Saudan, Philippe. The sequence listing filed with the application follows.

SEQUENCE LISTING (15 sequences)

SEQ ID NO: 1 - protein, 5 aa, Homo sapiens
GAKDV

SEQ ID NO: 2 - protein, 4 aa, Homo sapiens
KKKK

SEQ ID NO: 3 - protein, 16 aa, Homo sapiens
YRGDTIGEGQQHHLGG

SEQ ID NO: 4 - protein, 8 aa, Homo sapiens
NQEQVSPL

SEQ ID NO: 5 - protein, 6 aa, Homo sapiens
LIKMKP

SEQ ID NO: 6 - protein, 6 aa, Homo sapiens
NFKSQL

SEQ ID NO: 7 - protein, 8 aa, Homo sapiens
  MOD_RES (1)..(1): ACETYLATION
GPLALTAL

SEQ ID NO: 8 - protein, 6 aa, Homo sapiens
  MOD_RES (1)..(1): ACETYLATION
  MOD_RES (6)..(6): AMIDATION
PFELRA

SEQ ID NO: 9 - protein, 5 aa, Homo sapiens
  MOD_RES (4)..(4): AMIDATION
ZAAFA

SEQ ID NO: 10 - protein, 8 aa, Homo sapiens
GPLGIAGP

SEQ ID NO: 11 - protein, 8 aa, Homo sapiens
PHYGRSGG

SEQ ID NO: 12 - protein, 9 aa, Homo sapiens
PGSGRSASG

SEQ ID NO: 13 - protein, 4 aa, Homo sapiens
YKNR

SEQ ID NO: 14 - protein, 46 aa, Artificial Sequence
  Synthetic fusion protein
NQEQVSPLYKNRSVSEIQLMHNLGKHLNSMERVEWLRKKLQDVHNF

SEQ ID NO: 15 - protein, 42 aa, Artificial Sequence
  Synthetic fusion protein
NQEQVSPLSVSEIQLMHNLGKHLNSMERVEWLRKKLQDVHNF